European Patent Application EP 4 502 157 A1, published February 5, 2025. Title: SINGLE-STRANDED POLYNUCLEOTIDE AND USE THEREOF IN GENOME EDITING. Applicant: 国立研究開発法人産業技術総合研究所. Application JP. The sequence listing filed with the application follows.

SEQUENCE LISTING (41 sequences)

SEQ ID NO: 1 - DNA, 20 bp, synthetic construct
  source 1..20: mol_type = other DNA
cccgaccacatgaagcagca

SEQ ID NO: 2 - DNA, 40 bp, synthetic construct
  source 1..40: mol_type = other DNA
cagccgctaccccgaccacatgaagcagcacgacttcttc

SEQ ID NO: 3 - DNA, 60 bp, synthetic construct
  source 1..60: mol_type = other DNA
tgcagtgcttcagccgctaccccgaccacatgaagcagcacgacttcttcaagtccgcca

SEQ ID NO: 4 - DNA, 70 bp, synthetic construct
  source 1..70: mol_type = other DNA
cggcgtgcagtgcttcagccgctaccccgaccacatgaagcagcacgacttcttcaagtccgccatgccc

SEQ ID NO: 5 - DNA, 80 bp, synthetic construct
  source 1..80: mol_type = other DNA
acctacggcgtgcagtgcttcagccgctaccccgaccacatgaagcagcacgacttcttcaagtccgccatgcccgaagg

SEQ ID NO: 6 - DNA, 90 bp, synthetic construct
  source 1..90: mol_type = other DNA
ccctgacctacggcgtgcagtgcttcagccgctaccccgaccacatgaagcagcacgacttcttcaagtccgccatgcccgaaggctacg

SEQ ID NO: 7 - DNA, 100 bp, synthetic construct
  source 1..100: mol_type = other DNA
gaccaccctgacctacggcgtgcagtgcttcagccgctaccccgaccacatgaagcagcacgacttcttcaagtccgccatgcccgaaggctacgtccag

SEQ ID NO: 8 - DNA, 120 bp, synthetic construct
  source 1..120: mol_type = other DNA
ccaccctcgtgaccaccctgacctacggcgtgcagtgcttcagccgctaccccgaccacatgaagcagcacgacttcttcaagtccgccatgcccgaaggctacgtccaggagcgcacca

SEQ ID NO: 9 - DNA, 20 bp, synthetic construct
  modified_base 1: mod_base = OTHER; note = 2'-O,4'-C-methylene bridged nucleoside
  modified_base 3: mod_base = OTHER; note = 2'-O,4'-C-methylene bridged nucleoside
  modified_base 5: mod_base = OTHER; note = 2'-O,4'-C-methylene bridged nucleoside
  modified_base 7: mod_base = OTHER; note = 2'-O,4'-C-methylene bridged nucleoside
  modified_base 9: mod_base = OTHER; note = 2'-O,4'-C-methylene bridged nucleoside
  modified_base 12: mod_base = OTHER; note = 2'-O,4'-C-methylene bridged nucleoside
  modified_base 14: mod_base = OTHER; note = 2'-O,4'-C-methylene bridged nucleoside
  modified_base 16: mod_base = OTHER; note = 2'-O,4'-C-methylene bridged nucleoside
  modified_base 18: mod_base = OTHER; note = 2'-O,4'-C-methylene bridged nucleoside
  modified_base 20: mod_base = OTHER; note = 2'-O,4'-C-methylene bridged nucleoside
  modified_base 1: mod_base = m5c
  modified_base 3: mod_base = m5c
  modified_base 7: mod_base = m5c
  modified_base 9: mod_base = m5c
  modified_base 16: mod_base = m5c
  source 1..20: mol_type = other DNA
cccgaccacatgaagcagca

SEQ ID NO: 10 - DNA, 40 bp, synthetic construct; identical to SEQ ID NO: 2
  modified_base 1: mod_base = OTHER; note = 2'-O,4'-C-methylene bridged nucleoside
  modified_base 3: mod_base = OTHER; note = 2'-O,4'-C-methylene bridged nucleoside
  modified_base 5: mod_base = OTHER; note = 2'-O,4'-C-methylene bridged nucleoside
  modified_base 7: mod_base = OTHER; note = 2'-O,4'-C-methylene bridged nucleoside
  modified_base 9: mod_base = OTHER; note = 2'-O,4'-C-methylene bridged nucleoside
  modified_base 32: mod_base = OTHER; note = 2'-O,4'-C-methylene bridged nucleoside
  modified_base 34: mod_base = OTHER; note = 2'-O,4'-C-methylene bridged nucleoside
  modified_base 36: mod_base = OTHER; note = 2'-O,4'-C-methylene bridged nucleoside
  modified_base 38: mod_base = OTHER; note = 2'-O,4'-C-methylene bridged nucleoside
  modified_base 40: mod_base = OTHER; note = 2'-O,4'-C-methylene bridged nucleoside
  modified_base 1: mod_base = m5c
  modified_base 5: mod_base = m5c
  modified_base 7: mod_base = m5c
  modified_base 34: mod_base = m5c
  modified_base 40: mod_base = m5c
  source 1..40: mol_type = other DNA

SEQ ID NO: 11 - DNA, 60 bp, synthetic construct; identical to SEQ ID NO: 3
  modified_base 1: mod_base = OTHER; note = 2'-O,4'-C-methylene bridged nucleoside
  modified_base 3: mod_base = OTHER; note = 2'-O,4'-C-methylene bridged nucleoside
  modified_base 5: mod_base = OTHER; note = 2'-O,4'-C-methylene bridged nucleoside
  modified_base 7: mod_base = OTHER; note = 2'-O,4'-C-methylene bridged nucleoside
  modified_base 9: mod_base = OTHER; note = 2'-O,4'-C-methylene bridged nucleoside
  modified_base 52: mod_base = OTHER; note = 2'-O,4'-C-methylene bridged nucleoside
  modified_base 54: mod_base = OTHER; note = 2'-O,4'-C-methylene bridged nucleoside
  modified_base 56: mod_base = OTHER; note = 2'-O,4'-C-methylene bridged nucleoside
  modified_base 58: mod_base = OTHER; note = 2'-O,4'-C-methylene bridged nucleoside
  modified_base 60: mod_base = OTHER; note = 2'-O,4'-C-methylene bridged nucleoside
  modified_base 3: mod_base = m5c
  modified_base 56: mod_base = m5c
  modified_base 58: mod_base = m5c
  source 1..60: mol_type = other DNA

SEQ ID NO: 12 - DNA, 60 bp, synthetic construct; identical to SEQ ID NO: 3
  modified_base 1: mod_base = OTHER; note = 2'-O,4'-C-methylene bridged nucleoside
  modified_base 3: mod_base = OTHER; note = 2'-O,4'-C-methylene bridged nucleoside
  modified_base 5: mod_base = OTHER; note = 2'-O,4'-C-methylene bridged nucleoside
  modified_base 7: mod_base = OTHER; note = 2'-O,4'-C-methylene bridged nucleoside
  modified_base 9: mod_base = OTHER; note = 2'-O,4'-C-methylene bridged nucleoside
  modified_base 11: mod_base = OTHER; note = 2'-O,4'-C-methylene bridged nucleoside
  modified_base 50: mod_base = OTHER; note = 2'-O,4'-C-methylene bridged nucleoside
  modified_base 52: mod_base = OTHER; note = 2'-O,4'-C-methylene bridged nucleoside
  modified_base 54: mod_base = OTHER; note = 2'-O,4'-C-methylene bridged nucleoside
  modified_base 56: mod_base = OTHER; note = 2'-O,4'-C-methylene bridged nucleoside
  modified_base 58: mod_base = OTHER; note = 2'-O,4'-C-methylene bridged nucleoside
  modified_base 60: mod_base = OTHER; note = 2'-O,4'-C-methylene bridged nucleoside
  modified_base 3: mod_base = m5c
  modified_base 11: mod_base = m5c
  modified_base 50: mod_base = m5c
  modified_base 56: mod_base = m5c
  modified_base 58: mod_base = m5c
  source 1..60: mol_type = other DNA

SEQ ID NO: 13 - DNA, 70 bp, synthetic construct; identical to SEQ ID NO: 4
  modified_base 3: mod_base = OTHER; note = 2'-O,4'-C-methylene bridged nucleoside
  modified_base 5: mod_base = OTHER; note = 2'-O,4'-C-methylene bridged nucleoside
  modified_base 7: mod_base = OTHER; note = 2'-O,4'-C-methylene bridged nucleoside
  modified_base 9: mod_base = OTHER; note = 2'-O,4'-C-methylene bridged nucleoside
  modified_base 62: mod_base = OTHER; note = 2'-O,4'-C-methylene bridged nucleoside
  modified_base 64: mod_base = OTHER; note = 2'-O,4'-C-methylene bridged nucleoside
  modified_base 66: mod_base = OTHER; note = 2'-O,4'-C-methylene bridged nucleoside
  modified_base 68: mod_base = OTHER; note = 2'-O,4'-C-methylene bridged nucleoside
  modified_base 64: mod_base = m5c
  modified_base 68: mod_base = m5c
  source 1..70: mol_type = other DNA

SEQ ID NO: 14 - DNA, 70 bp, synthetic construct; identical to SEQ ID NO: 4
  modified_base 3: mod_base = OTHER; note = 2'-O,4'-C-methylene bridged nucleoside
  modified_base 5: mod_base = OTHER; note = 2'-O,4'-C-methylene bridged nucleoside
  modified_base 7: mod_base = OTHER; note = 2'-O,4'-C-methylene bridged nucleoside
  modified_base 9: mod_base = OTHER; note = 2'-O,4'-C-methylene bridged nucleoside
  modified_base 15: mod_base = OTHER; note = 2'-O,4'-C-methylene bridged nucleoside
  modified_base 56: mod_base = OTHER; note = 2'-O,4'-C-methylene bridged nucleoside
  modified_base 62: mod_base = OTHER; note = 2'-O,4'-C-methylene bridged nucleoside
  modified_base 64: mod_base = OTHER; note = 2'-O,4'-C-methylene bridged nucleoside
  modified_base 66: mod_base = OTHER; note = 2'-O,4'-C-methylene bridged nucleoside
  modified_base 68: mod_base = OTHER; note = 2'-O,4'-C-methylene bridged nucleoside
  modified_base 64: mod_base = m5c
  modified_base 68: mod_base = m5c
  source 1..70: mol_type = other DNA

SEQ ID NO: 15 - DNA, 70 bp, synthetic construct; identical to SEQ ID NO: 4
  modified_base 5: mod_base = OTHER; note = 2'-O,4'-C-methylene bridged nucleoside
  modified_base 7: mod_base = OTHER; note = 2'-O,4'-C-methylene bridged nucleoside
  modified_base 9: mod_base = OTHER; note = 2'-O,4'-C-methylene bridged nucleoside
  modified_base 62: mod_base = OTHER; note = 2'-O,4'-C-methylene bridged nucleoside
  modified_base 64: mod_base = OTHER; note = 2'-O,4'-C-methylene bridged nucleoside
  modified_base 66: mod_base = OTHER; note = 2'-O,4'-C-methylene bridged nucleoside
  modified_base 64: mod_base = m5c
  source 1..70: mol_type = other DNA

SEQ ID NO: 16 - DNA, 70 bp, synthetic construct; identical to SEQ ID NO: 4
  modified_base 7: mod_base = OTHER; note = 2'-O,4'-C-methylene bridged nucleoside
  modified_base 9: mod_base = OTHER; note = 2'-O,4'-C-methylene bridged nucleoside
  modified_base 62: mod_base = OTHER; note = 2'-O,4'-C-methylene bridged nucleoside
  modified_base 64: mod_base = OTHER; note = 2'-O,4'-C-methylene bridged nucleoside
  modified_base 64: mod_base = m5c
  source 1..70: mol_type = other DNA

SEQ ID NO: 17 - DNA, 70 bp, synthetic construct; identical to SEQ ID NO: 4
  modified_base 9: mod_base = OTHER; note = 2'-O,4'-C-methylene bridged nucleoside
  modified_base 62: mod_base = OTHER; note = 2'-O,4'-C-methylene bridged nucleoside
  source 1..70: mol_type = other DNA

SEQ ID NO: 18 - DNA, 70 bp, synthetic construct; identical to SEQ ID NO: 4
  modified_base 1: mod_base = OTHER; note = 2'-O,4'-C-methylene bridged nucleoside
  modified_base 3: mod_base = OTHER; note = 2'-O,4'-C-methylene bridged nucleoside
  modified_base 5: mod_base = OTHER; note = 2'-O,4'-C-methylene bridged nucleoside
  modified_base 7: mod_base = OTHER; note = 2'-O,4'-C-methylene bridged nucleoside
  modified_base 9: mod_base = OTHER; note = 2'-O,4'-C-methylene bridged nucleoside
  modified_base 62: mod_base = OTHER; note = 2'-O,4'-C-methylene bridged nucleoside
  modified_base 64: mod_base = OTHER; note = 2'-O,4'-C-methylene bridged nucleoside
  modified_base 66: mod_base = OTHER; note = 2'-O,4'-C-methylene bridged nucleoside
  modified_base 68: mod_base = OTHER; note = 2'-O,4'-C-methylene bridged nucleoside
  modified_base 70: mod_base = OTHER; note = 2'-O,4'-C-methylene bridged nucleoside
  modified_base 1: mod_base = m5c
  modified_base 64: mod_base = m5c
  modified_base 68: mod_base = m5c
  modified_base 70: mod_base = m5c
  source 1..70: mol_type = other DNA

SEQ ID NO: 19 - DNA, 70 bp, synthetic construct; identical to SEQ ID NO: 4
  modified_base 1: mod_base = OTHER; note = 2'-O,4'-C-methylene bridged nucleoside
  modified_base 3: mod_base = OTHER; note = 2'-O,4'-C-methylene bridged nucleoside
  modified_base 5: mod_base = OTHER; note = 2'-O,4'-C-methylene bridged nucleoside
  modified_base 7: mod_base = OTHER; note = 2'-O,4'-C-methylene bridged nucleoside
  modified_base 9: mod_base = OTHER; note = 2'-O,4'-C-methylene bridged nucleoside
  modified_base 15: mod_base = OTHER; note = 2'-O,4'-C-methylene bridged nucleoside
  modified_base 56: mod_base = OTHER; note = 2'-O,4'-C-methylene bridged nucleoside
  modified_base 62: mod_base = OTHER; note = 2'-O,4'-C-methylene bridged nucleoside
  modified_base 64: mod_base = OTHER; note = 2'-O,4'-C-methylene bridged nucleoside
  modified_base 66: mod_base = OTHER; note = 2'-O,4'-C-methylene bridged nucleoside
  modified_base 68: mod_base = OTHER; note = 2'-O,4'-C-methylene bridged nucleoside
  modified_base 70: mod_base = OTHER; note = 2'-O,4'-C-methylene bridged nucleoside
  modified_base 1: mod_base = m5c
  modified_base 64: mod_base = m5c
  modified_base 68: mod_base = m5c
  modified_base 70: mod_base = m5c
  source 1..70: mol_type = other DNA

SEQ ID NO: 20 - DNA, 80 bp, synthetic construct; identical to SEQ ID NO: 5
  modified_base 1: mod_base = OTHER; note = 2'-O,4'-C-methylene bridged nucleoside
  modified_base 3: mod_base = OTHER; note = 2'-O,4'-C-methylene bridged nucleoside
  modified_base 5: mod_base = OTHER; note = 2'-O,4'-C-methylene bridged nucleoside
  modified_base 7: mod_base = OTHER; note = 2'-O,4'-C-methylene bridged nucleoside
  modified_base 9: mod_base = OTHER; note = 2'-O,4'-C-methylene bridged nucleoside
  modified_base 72: mod_base = OTHER; note = 2'-O,4'-C-methylene bridged nucleoside
  modified_base 74: mod_base = OTHER; note = 2'-O,4'-C-methylene bridged nucleoside
  modified_base 76: mod_base = OTHER; note = 2'-O,4'-C-methylene bridged nucleoside
  modified_base 78: mod_base = OTHER; note = 2'-O,4'-C-methylene bridged nucleoside
  modified_base 80: mod_base = OTHER; note = 2'-O,4'-C-methylene bridged nucleoside
  modified_base 3: mod_base = m5c
  modified_base 9: mod_base = m5c
  modified_base 74: mod_base = m5c
  source 1..80: mol_type = other DNA

SEQ ID NO: 21 - DNA, 80 bp, synthetic construct; identical to SEQ ID NO: 5
  modified_base 1: mod_base = OTHER; note = 2'-O,4'-C-methylene bridged nucleoside
  modified_base 3: mod_base = OTHER; note = 2'-O,4'-C-methylene bridged nucleoside
  modified_base 5: mod_base = OTHER; note = 2'-O,4'-C-methylene bridged nucleoside
  modified_base 7: mod_base = OTHER; note = 2'-O,4'-C-methylene bridged nucleoside
  modified_base 9: mod_base = OTHER; note = 2'-O,4'-C-methylene bridged nucleoside
  modified_base 39: mod_base = OTHER; note = 2'-O,4'-C-methylene bridged nucleoside
  modified_base 42: mod_base = OTHER; note = 2'-O,4'-C-methylene bridged nucleoside
  modified_base 72: mod_base = OTHER; note = 2'-O,4'-C-methylene bridged nucleoside
  modified_base 74: mod_base = OTHER; note = 2'-O,4'-C-methylene bridged nucleoside
  modified_base 76: mod_base = OTHER; note = 2'-O,4'-C-methylene bridged nucleoside
  modified_base 78: mod_base = OTHER; note = 2'-O,4'-C-methylene bridged nucleoside
  modified_base 80: mod_base = OTHER; note = 2'-O,4'-C-methylene bridged nucleoside
  modified_base 3: mod_base = m5c
  modified_base 9: mod_base = m5c
  modified_base 39: mod_base = m5c
  modified_base 74: mod_base = m5c
  source 1..80: mol_type = other DNA

SEQ ID NO: 22 - DNA, 80 bp, synthetic construct; identical to SEQ ID NO: 5
  modified_base 1: mod_base = OTHER; note = 2'-O,4'-C-methylene bridged nucleoside
  modified_base 3: mod_base = OTHER; note = 2'-O,4'-C-methylene bridged nucleoside
  modified_base 5: mod_base = OTHER; note = 2'-O,4'-C-methylene bridged nucleoside
  modified_base 7: mod_base = OTHER; note = 2'-O,4'-C-methylene bridged nucleoside
  modified_base 9: mod_base = OTHER; note = 2'-O,4'-C-methylene bridged nucleoside
  modified_base 11: mod_base = OTHER; note = 2'-O,4'-C-methylene bridged nucleoside
  modified_base 70: mod_base = OTHER; note = 2'-O,4'-C-methylene bridged nucleoside
  modified_base 72: mod_base = OTHER; note = 2'-O,4'-C-methylene bridged nucleoside
  modified_base 74: mod_base = OTHER; note = 2'-O,4'-C-methylene bridged nucleoside
  modified_base 76: mod_base = OTHER; note = 2'-O,4'-C-methylene bridged nucleoside
  modified_base 78: mod_base = OTHER; note = 2'-O,4'-C-methylene bridged nucleoside
  modified_base 80: mod_base = OTHER; note = 2'-O,4'-C-methylene bridged nucleoside
  modified_base 3: mod_base = m5c
  modified_base 9: mod_base = m5c
  modified_base 74: mod_base = m5c
  source 1..80: mol_type = other DNA

SEQ ID NO: 23 - DNA, 80 bp, synthetic construct; identical to SEQ ID NO: 5
  modified_base 1: mod_base = OTHER; note = 2'-O,4'-C-methylene bridged nucleoside
  modified_base 3: mod_base = OTHER; note = 2'-O,4'-C-methylene bridged nucleoside
  modified_base 5: mod_base = OTHER; note = 2'-O,4'-C-methylene bridged nucleoside
  modified_base 7: mod_base = OTHER; note = 2'-O,4'-C-methylene bridged nucleoside
  modified_base 9: mod_base = OTHER; note = 2'-O,4'-C-methylene bridged nucleoside
  modified_base 11: mod_base = OTHER; note = 2'-O,4'-C-methylene bridged nucleoside
  modified_base 35: mod_base = OTHER; note = 2'-O,4'-C-methylene bridged nucleoside
  modified_base 46: mod_base = OTHER; note = 2'-O,4'-C-methylene bridged nucleoside
  modified_base 70: mod_base = OTHER; note = 2'-O,4'-C-methylene bridged nucleoside
  modified_base 72: mod_base = OTHER; note = 2'-O,4'-C-methylene bridged nucleoside
  modified_base 74: mod_base = OTHER; note = 2'-O,4'-C-methylene bridged nucleoside
  modified_base 76: mod_base = OTHER; note = 2'-O,4'-C-methylene bridged nucleoside
  modified_base 78: mod_base = OTHER; note = 2'-O,4'-C-methylene bridged nucleoside
  modified_base 80: mod_base = OTHER; note = 2'-O,4'-C-methylene bridged nucleoside
  modified_base 3: mod_base = m5c
  modified_base 9: mod_base = m5c
  modified_base 46: mod_base = m5c
  modified_base 74: mod_base = m5c
  source 1..80: mol_type = other DNA

SEQ ID NO: 24 - DNA, 80 bp, synthetic construct; identical to SEQ ID NO: 5
  modified_base 1: mod_base = OTHER; note = 2'-O,4'-C-methylene bridged nucleoside
  modified_base 3: mod_base = OTHER; note = 2'-O,4'-C-methylene bridged nucleoside
  modified_base 5: mod_base = OTHER; note = 2'-O,4'-C-methylene bridged nucleoside
  modified_base 7: mod_base = OTHER; note = 2'-O,4'-C-methylene bridged nucleoside
  modified_base 9: mod_base = OTHER; note = 2'-O,4'-C-methylene bridged nucleoside
  modified_base 11: mod_base = OTHER; note = 2'-O,4'-C-methylene bridged nucleoside
  modified_base 30: mod_base = OTHER; note = 2'-O,4'-C-methylene bridged nucleoside
  modified_base 51: mod_base = OTHER; note = 2'-O,4'-C-methylene bridged nucleoside
  modified_base 70: mod_base = OTHER; note = 2'-O,4'-C-methylene bridged nucleoside
  modified_base 72: mod_base = OTHER; note = 2'-O,4'-C-methylene bridged nucleoside
  modified_base 74: mod_base = OTHER; note = 2'-O,4'-C-methylene bridged nucleoside
  modified_base 76: mod_base = OTHER; note = 2'-O,4'-C-methylene bridged nucleoside
  modified_base 78: mod_base = OTHER; note = 2'-O,4'-C-methylene bridged nucleoside
  modified_base 80: mod_base = OTHER; note = 2'-O,4'-C-methylene bridged nucleoside
  modified_base 3: mod_base = m5c
  modified_base 9: mod_base = m5c
  modified_base 30: mod_base = m5c
  modified_base 51: mod_base = m5c
  modified_base 74: mod_base = m5c
  source 1..80: mol_type = other DNA

SEQ ID NO: 25 - DNA, 80 bp, synthetic construct; identical to SEQ ID NO: 5
  modified_base 1: mod_base = OTHER; note = 2'-O,4'-C-methylene bridged nucleoside
  modified_base 3: mod_base = OTHER; note = 2'-O,4'-C-methylene bridged nucleoside
  modified_base 5: mod_base = OTHER; note = 2'-O,4'-C-methylene bridged nucleoside
  modified_base 7: mod_base = OTHER; note = 2'-O,4'-C-methylene bridged nucleoside
  modified_base 9: mod_base = OTHER; note = 2'-O,4'-C-methylene bridged nucleoside
  modified_base 11: mod_base = OTHER; note = 2'-O,4'-C-methylene bridged nucleoside
  modified_base 25: mod_base = OTHER; note = 2'-O,4'-C-methylene bridged nucleoside
  modified_base 56: mod_base = OTHER; note = 2'-O,4'-C-methylene bridged nucleoside
  modified_base 70: mod_base = OTHER; note = 2'-O,4'-C-methylene bridged nucleoside
  modified_base 72: mod_base = OTHER; note = 2'-O,4'-C-methylene bridged nucleoside
  modified_base 74: mod_base = OTHER; note = 2'-O,4'-C-methylene bridged nucleoside
  modified_base 76: mod_base = OTHER; note = 2'-O,4'-C-methylene bridged nucleoside
  modified_base 78: mod_base = OTHER; note = 2'-O,4'-C-methylene bridged nucleoside
  modified_base 80: mod_base = OTHER; note = 2'-O,4'-C-methylene bridged nucleoside
  modified_base 3: mod_base = m5c
  modified_base 9: mod_base = m5c
  modified_base 25: mod_base = m5c
  modified_base 74: mod_base = m5c
  source 1..80: mol_type = other DNA

SEQ ID NO: 26 - DNA, 80 bp, synthetic construct; identical to SEQ ID NO: 5
  modified_base 1: mod_base = OTHER; note = 2'-O,4'-C-methylene bridged nucleoside
  modified_base 3: mod_base = OTHER; note = 2'-O,4'-C-methylene bridged nucleoside
  modified_base 5: mod_base = OTHER; note = 2'-O,4'-C-methylene bridged nucleoside
  modified_base 7: mod_base = OTHER; note = 2'-O,4'-C-methylene bridged nucleoside
  modified_base 9: mod_base = OTHER; note = 2'-O,4'-C-methylene bridged nucleoside
  modified_base 11: mod_base = OTHER; note = 2'-O,4'-C-methylene bridged nucleoside
  modified_base 20: mod_base = OTHER; note = 2'-O,4'-C-methylene bridged nucleoside
  modified_base 61: mod_base = OTHER; note = 2'-O,4'-C-methylene bridged nucleoside
  modified_base 70: mod_base = OTHER; note = 2'-O,4'-C-methylene bridged nucleoside
  modified_base 72: mod_base = OTHER; note = 2'-O,4'-C-methylene bridged nucleoside
  modified_base 74: mod_base = OTHER; note = 2'-O,4'-C-methylene bridged nucleoside
  modified_base 76: mod_base = OTHER; note = 2'-O,4'-C-methylene bridged nucleoside
  modified_base 78: mod_base = OTHER; note = 2'-O,4'-C-methylene bridged nucleoside
  modified_base 80: mod_base = OTHER; note = 2'-O,4'-C-methylene bridged nucleoside
  modified_base 3: mod_base = m5c
  modified_base 9: mod_base = m5c
  modified_base 74: mod_base = m5c
  source 1..80: mol_type = other DNA

SEQ ID NO: 27 - DNA, 80 bp, synthetic construct; identical to SEQ ID NO: 5
  modified_base 1: mod_base = OTHER; note = 2'-O,4'-C-methylene bridged nucleoside
  modified_base 3: mod_base = OTHER; note = 2'-O,4'-C-methylene bridged nucleoside
  modified_base 5: mod_base = OTHER; note = 2'-O,4'-C-methylene bridged nucleoside
  modified_base 7: mod_base = OTHER; note = 2'-O,4'-C-methylene bridged nucleoside
  modified_base 9: mod_base = OTHER; note = 2'-O,4'-C-methylene bridged nucleoside
  modified_base 11: mod_base = OTHER; note = 2'-O,4'-C-methylene bridged nucleoside
  modified_base 15: mod_base = OTHER; note = 2'-O,4'-C-methylene bridged nucleoside
  modified_base 66: mod_base = OTHER; note = 2'-O,4'-C-methylene bridged nucleoside
  modified_base 70: mod_base = OTHER; note = 2'-O,4'-C-methylene bridged nucleoside
  modified_base 72: mod_base = OTHER; note = 2'-O,4'-C-methylene bridged nucleoside
  modified_base 74: mod_base = OTHER; note = 2'-O,4'-C-methylene bridged nucleoside
  modified_base 76: mod_base = OTHER; note = 2'-O,4'-C-methylene bridged nucleoside
  modified_base 78: mod_base = OTHER; note = 2'-O,4'-C-methylene bridged nucleoside
  modified_base 80: mod_base = OTHER; note = 2'-O,4'-C-methylene bridged nucleoside
  modified_base 3: mod_base = m5c
  modified_base 9: mod_base = m5c
  modified_base 66: mod_base = m5c
  modified_base 74: mod_base = m5c
  source 1..80: mol_type = other DNA

SEQ ID NO: 28 - DNA, 80 bp, synthetic construct; identical to SEQ ID NO: 5
  modified_base 1: mod_base = OTHER; note = 2'-O,4'-C-methylene bridged nucleoside
  modified_base 3: mod_base = OTHER; note = 2'-O,4'-C-methylene bridged nucleoside
  modified_base 5: mod_base = OTHER; note = 2'-O,4'-C-methylene bridged nucleoside
  modified_base 7: mod_base = OTHER; note = 2'-O,4'-C-methylene bridged nucleoside
  modified_base 9: mod_base = OTHER; note = 2'-O,4'-C-methylene bridged nucleoside
  modified_base 11: mod_base = OTHER; note = 2'-O,4'-C-methylene bridged nucleoside
  modified_base 39: mod_base = OTHER; note = 2'-O,4'-C-methylene bridged nucleoside
  modified_base 42: mod_base = OTHER; note = 2'-O,4'-C-methylene bridged nucleoside
  modified_base 70: mod_base = OTHER; note = 2'-O,4'-C-methylene bridged nucleoside
  modified_base 72: mod_base = OTHER; note = 2'-O,4'-C-methylene bridged nucleoside
  modified_base 74: mod_base = OTHER; note = 2'-O,4'-C-methylene bridged nucleoside
  modified_base 76: mod_base = OTHER; note = 2'-O,4'-C-methylene bridged nucleoside
  modified_base 78: mod_base = OTHER; note = 2'-O,4'-C-methylene bridged nucleoside
  modified_base 80: mod_base = OTHER; note = 2'-O,4'-C-methylene bridged nucleoside
  modified_base 3: mod_base = m5c
  modified_base 9: mod_base = m5c
  modified_base 39: mod_base = m5c
  modified_base 74: mod_base = m5c
  source 1..80: mol_type = other DNA

SEQ ID NO: 29 - DNA, 80 bp, synthetic construct; identical to SEQ ID NO: 5
  modified_base 1: mod_base = OTHER; note = 2'-O,4'-C-methylene bridged nucleoside
  modified_base 3: mod_base = OTHER; note = 2'-O,4'-C-methylene bridged nucleoside
  modified_base 5: mod_base = OTHER; note = 2'-O,4'-C-methylene bridged nucleoside
  modified_base 7: mod_base = OTHER; note = 2'-O,4'-C-methylene bridged nucleoside
  modified_base 9: mod_base = OTHER; note = 2'-O,4'-C-methylene bridged nucleoside
  modified_base 11: mod_base = OTHER; note = 2'-O,4'-C-methylene bridged nucleoside
  modified_base 13: mod_base = OTHER; note = 2'-O,4'-C-methylene bridged nucleoside
  modified_base 68: mod_base = OTHER; note = 2'-O,4'-C-methylene bridged nucleoside
  modified_base 70: mod_base = OTHER; note = 2'-O,4'-C-methylene bridged nucleoside
  modified_base 72: mod_base = OTHER; note = 2'-O,4'-C-methylene bridged nucleoside
  modified_base 74: mod_base = OTHER; note = 2'-O,4'-C-methylene bridged nucleoside
  modified_base 76: mod_base = OTHER; note = 2'-O,4'-C-methylene bridged nucleoside
  modified_base 78: mod_base = OTHER; note = 2'-O,4'-C-methylene bridged nucleoside
  modified_base 80: mod_base = OTHER; note = 2'-O,4'-C-methylene bridged nucleoside
  modified_base 3: mod_base = m5c
  modified_base 9: mod_base = m5c
  modified_base 13: mod_base = m5c
  modified_base 68: mod_base = m5c
  modified_base 74: mod_base = m5c
  source 1..80: mol_type = other DNA

SEQ ID NO: 30 - DNA, 80 bp, synthetic construct; identical to SEQ ID NO: 5
  modified_base 11: mod_base = OTHER; note = 2'-O,4'-C-methylene bridged nucleoside
  modified_base 13: mod_base = OTHER; note = 2'-O,4'-C-methylene bridged nucleoside
  modified_base 15: mod_base = OTHER; note = 2'-O,4'-C-methylene bridged nucleoside
  modified_base 17: mod_base = OTHER; note = 2'-O,4'-C-methylene bridged nucleoside
  modified_base 19: mod_base = OTHER; note = 2'-O,4'-C-methylene bridged nucleoside
  modified_base 21: mod_base = OTHER; note = 2'-O,4'-C-methylene bridged nucleoside
  modified_base 60: mod_base = OTHER; note = 2'-O,4'-C-methylene bridged nucleoside
  modified_base 62: mod_base = OTHER; note = 2'-O,4'-C-methylene bridged nucleoside
  modified_base 64: mod_base = OTHER; note = 2'-O,4'-C-methylene bridged nucleoside
  modified_base 66: mod_base = OTHER; note = 2'-O,4'-C-methylene bridged nucleoside
  modified_base 68: mod_base = OTHER; note = 2'-O,4'-C-methylene bridged nucleoside
  modified_base 70: mod_base = OTHER; note = 2'-O,4'-C-methylene bridged nucleoside
  modified_base 13: mod_base = m5c
  modified_base 21: mod_base = m5c
  modified_base 60: mod_base = m5c
  modified_base 66: mod_base = m5c
  modified_base 68: mod_base = m5c
  source 1..80: mol_type = other DNA

SEQ ID NO: 31 - DNA, 80 bp, synthetic construct; identical to SEQ ID NO: 5
  modified_base 1: mod_base = OTHER; note = 2'-O,4'-C-methylene bridged nucleoside
  modified_base 3: mod_base = OTHER; note = 2'-O,4'-C-methylene bridged nucleoside
  modified_base 5: mod_base = OTHER; note = 2'-O,4'-C-methylene bridged nucleoside
  modified_base 76: mod_base = OTHER; note = 2'-O,4'-C-methylene bridged nucleoside
  modified_base 78: mod_base = OTHER; note = 2'-O,4'-C-methylene bridged nucleoside
  modified_base 80: mod_base = OTHER; note = 2'-O,4'-C-methylene bridged nucleoside
  modified_base 3: mod_base = m5c
  source 1..80: mol_type = other DNA

SEQ ID NO: 32 - DNA, 80 bp, synthetic construct; identical to SEQ ID NO: 5
  modified_base 1: mod_base = OTHER; note = 2'-O,4'-C-methylene bridged nucleoside
  modified_base 3: mod_base = OTHER; note = 2'-O,4'-C-methylene bridged nucleoside
  modified_base 5: mod_base = OTHER; note = 2'-O,4'-C-methylene bridged nucleoside
  modified_base 7: mod_base = OTHER; note = 2'-O,4'-C-methylene bridged nucleoside
  modified_base 74: mod_base = OTHER; note = 2'-O,4'-C-methylene bridged nucleoside
  modified_base 76: mod_base = OTHER; note = 2'-O,4'-C-methylene bridged nucleoside
  modified_base 78: mod_base = OTHER; note = 2'-O,4'-C-methylene bridged nucleoside
  modified_base 80: mod_base = OTHER; note = 2'-O,4'-C-methylene bridged nucleoside
  modified_base 3: mod_base = m5c
  modified_base 74: mod_base = m5c
  source 1..80: mol_type = other DNA

SEQ ID NO: 33 - DNA, 90 bp, synthetic construct; identical to SEQ ID NO: 6
  modified_base 1: mod_base = OTHER; note = 2'-O,4'-C-methylene bridged nucleoside
  modified_base 3: mod_base = OTHER; note = 2'-O,4'-C-methylene bridged nucleoside
  modified_base 5: mod_base = OTHER; note = 2'-O,4'-C-methylene bridged nucleoside
  modified_base 7: mod_base = OTHER; note = 2'-O,4'-C-methylene bridged nucleoside
  modified_base 9: mod_base = OTHER; note = 2'-O,4'-C-methylene bridged nucleoside
  modified_base 82: mod_base = OTHER; note = 2'-O,4'-C-methylene bridged nucleoside
  modified_base 84: mod_base = OTHER; note = 2'-O,4'-C-methylene bridged nucleoside
  modified_base 86: mod_base = OTHER; note = 2'-O,4'-C-methylene bridged nucleoside
  modified_base 88: mod_base = OTHER; note = 2'-O,4'-C-methylene bridged nucleoside
  modified_base 90: mod_base = OTHER; note = 2'-O,4'-C-methylene bridged nucleoside
  modified_base 1: mod_base = m5c
  modified_base 3: mod_base = m5c
  modified_base 7: mod_base = m5c
  modified_base 86: mod_base = m5c
  source 1..90: mol_type = other DNA

SEQ ID NO: 34 - DNA, 100 bp, synthetic construct; identical to SEQ ID NO: 7
  modified_base 1: mod_base = OTHER; note = 2'-O,4'-C-methylene bridged nucleoside
  modified_base 3: mod_base = OTHER; note = 2'-O,4'-C-methylene bridged nucleoside
  modified_base 5: mod_base = OTHER; note = 2'-O,4'-C-methylene bridged nucleoside
  modified_base 7: mod_base = OTHER; note = 2'-O,4'-C-methylene bridged nucleoside
  modified_base 9: mod_base = OTHER; note = 2'-O,4'-C-methylene bridged nucleoside
  modified_base 92: mod_base = OTHER; note = 2'-O,4'-C-methylene bridged nucleoside
  modified_base 94: mod_base = OTHER; note = 2'-O,4'-C-methylene bridged nucleoside
  modified_base 96: mod_base = OTHER; note = 2'-O,4'-C-methylene bridged nucleoside
  modified_base 98: mod_base = OTHER; note = 2'-O,4'-C-methylene bridged nucleoside
  modified_base 100: mod_base = OTHER; note = 2'-O,4'-C-methylene bridged nucleoside
  modified_base 3: mod_base = m5c
  modified_base 7: mod_base = m5c
  modified_base 94: mod_base = m5c
  modified_base 98: mod_base = m5c
  source 1..100: mol_type = other DNA

SEQ ID NO: 35 - DNA, 100 bp, synthetic construct; identical to SEQ ID NO: 7
  modified_base 11: mod_base = OTHER; note = 2'-O,4'-C-methylene bridged nucleoside
  modified_base 13: mod_base = OTHER; note = 2'-O,4'-C-methylene bridged nucleoside
  modified_base 15: mod_base = OTHER; note = 2'-O,4'-C-methylene bridged nucleoside
  modified_base 17: mod_base = OTHER; note = 2'-O,4'-C-methylene bridged nucleoside
  modified_base 19: mod_base = OTHER; note = 2'-O,4'-C-methylene bridged nucleoside
  modified_base 82: mod_base = OTHER; note = 2'-O,4'-C-methylene bridged nucleoside
  modified_base 84: mod_base = OTHER; note = 2'-O,4'-C-methylene bridged nucleoside
  modified_base 86: mod_base = OTHER; note = 2'-O,4'-C-methylene bridged nucleoside
  modified_base 88: mod_base = OTHER; note = 2'-O,4'-C-methylene bridged nucleoside
  modified_base 90: mod_base = OTHER; note = 2'-O,4'-C-methylene bridged nucleoside
  modified_base 13: mod_base = m5c
  modified_base 19: mod_base = m5c
  modified_base 84: mod_base = m5c
  source 1..100: mol_type = other DNA

SEQ ID NO: 36 - DNA, 120 bp, synthetic construct; identical to SEQ ID NO: 8
  modified_base 1: mod_base = OTHER; note = 2'-O,4'-C-methylene bridged nucleoside
  modified_base 3: mod_base = OTHER; note = 2'-O,4'-C-methylene bridged nucleoside
  modified_base 5: mod_base = OTHER; note = 2'-O,4'-C-methylene bridged nucleoside
  modified_base 7: mod_base = OTHER; note = 2'-O,4'-C-methylene bridged nucleoside
  modified_base 9: mod_base = OTHER; note = 2'-O,4'-C-methylene bridged nucleoside
  modified_base 112: mod_base = OTHER; note = 2'-O,4'-C-methylene bridged nucleoside
  modified_base 114: mod_base = OTHER; note = 2'-O,4'-C-methylene bridged nucleoside
  modified_base 116: mod_base = OTHER; note = 2'-O,4'-C-methylene bridged nucleoside
  modified_base 118: mod_base = OTHER; note = 2'-O,4'-C-methylene bridged nucleoside
  modified_base 120: mod_base = OTHER; note = 2'-O,4'-C-methylene bridged nucleoside
  modified_base 1: mod_base = m5c
  modified_base 5: mod_base = m5c
  modified_base 114: mod_base = m5c
  modified_base 116: mod_base = m5c
  modified_base 118: mod_base = m5c
  source 1..120: mol_type = other DNA

SEQ ID NO: 37 - DNA, 731 bp, synthetic construct
  misc_feature 1..731: note = polynucleotide encoding modified GFP with eight nucleotide insertion
  source 1..731: mol_type = other DNA
atggtgagcaagggcgaggagctgttcaccggggtggtgcccatcctggtcgagctggacggcgacgtaaacggccacaagttcagcgtgtccggcgagggcgagggcgatgccacctacggcaagctgaccctgaagttcatctgcaccaccggcaagctgcccgtgccctggcccaccctcgtgaccaccctgacctacggcgtgcagtgcttcagccgctaccccgaccacacggccagctgaagcagcacgacttcttcaagtccgccatgcccgaaggctacgtccaggagcgcaccatcttcttcaaggacgacggcaactacaagacccgcgccgaggtgaagttcgagggcgacaccctggtgaaccgcatcgagctgaagggcatcgacttcaaggaggacggcaacatcctggggcacaagctggagtacaactacaacagccacaacgtctatatcatggccgacaagcagaagaacggcatcaaggtgaacttcaagatccgccacaacatcgaggacggcagcgtgcagctcgccgaccactaccagcagaacacccccatcggcgacggccccgtgctgctgcccgacaaccactacctgagcacccagtccgccctgagcaaagaccccaacgagaagcgcgatcacatggtcctgctggagttcgtgaccgccgccgggatcactctcggcatggacgagctgtacaagtactag

SEQ ID NO: 38 - DNA, 723 bp, synthetic construct
  misc_feature 1..723: note = polynucleotide encoding modified GFP with one nucleotide substitution
  source 1..723: mol_type = other DNA
atggtgagcaagggcgaggagctgttcaccggggtggtgcccatcctggtcgagctggacggcgacgtaaacggccacaagttcagcgtgtccggcgagggcgagggcgatgccacctacggcaagctgaccctgaagttcatctgcaccaccggcaagctgcccgtgccctggcccaccctcgtgaccaccctgacctacggcgtgcagtgcttcagccgctaccccgaccacatgtagcagcacgacttcttcaagtccgccatgcccgaaggctacgtccaggagcgcaccatcttcttcaaggacgacggcaactacaagacccgcgccgaggtgaagttcgagggcgacaccctggtgaaccgcatcgagctgaagggcatcgacttcaaggaggacggcaacatcctggggcacaagctggagtacaactacaacagccacaacgtctatatcatggccgacaagcagaagaacggcatcaaggtgaacttcaagatccgccacaacatcgaggacggcagcgtgcagctcgccgaccactaccagcagaacacccccatcggcgacggccccgtgctgctgcccgacaaccactacctgagcacccagtccgccctgagcaaagaccccaacgagaagcgcgatcacatggtcctgctggagttcgtgaccgccgccgggatcactctcggcatggacgagctgtacaagtactag

SEQ ID NO: 39 - DNA, 70 bp, synthetic construct
  source 1..70: mol_type = other DNA
taggtcagggtggtcacgagggtgggccagggcacgggcagcttgccggtggtgcagatgaacttcaggg

SEQ ID NO: 40 - DNA, 70 bp, synthetic construct
  source 1..70: mol_type = other DNA
tcacctcggcgcgggtcttgtagttgccgtcgtccttgaagaagatggtgcgctcctggacgtagccttc

SEQ ID NO: 41 - DNA, 90 bp, synthetic construct; identical to SEQ ID NO: 6
  modified_base 11: mod_base = OTHER; note = 2'-O,4'-C-methylene bridged nucleoside
  modified_base 13: mod_base = OTHER; note = 2'-O,4'-C-methylene bridged nucleoside
  modified_base 15: mod_base = OTHER; note = 2'-O,4'-C-methylene bridged nucleoside
  modified_base 17: mod_base = OTHER; note = 2'-O,4'-C-methylene bridged nucleoside
  modified_base 19: mod_base = OTHER; note = 2'-O,4'-C-methylene bridged nucleoside
  modified_base 25: mod_base = OTHER; note = 2'-O,4'-C-methylene bridged nucleoside
  modified_base 66: mod_base = OTHER; note = 2'-O,4'-C-methylene bridged nucleoside
  modified_base 72: mod_base = OTHER; note = 2'-O,4'-C-methylene bridged nucleoside
  modified_base 74: mod_base = OTHER; note = 2'-O,4'-C-methylene bridged nucleoside
  modified_base 76: mod_base = OTHER; note = 2'-O,4'-C-methylene bridged nucleoside
  modified_base 78: mod_base = OTHER; note = 2'-O,4'-C-methylene bridged nucleoside
  modified_base 80: mod_base = OTHER; note = 2'-O,4'-C-methylene bridged nucleoside
  modified_base 11: mod_base = m5c
  modified_base 74: mod_base = m5c
  modified_base 78: mod_base = m5c
  modified_base 80: mod_base = m5c
  source 1..90: mol_type = other DNA